European Patent Application EP 4 198 053 A1, published June 21, 2023. Title: LMNA gene expression for treatment of laminopathies. Applicant: Universitätsklinikum Hamburg-Eppendorf. The sequence listing filed with the application follows.

SEQUENCE LISTING (19 sequences)

SEQ ID NO: 1 - protein, 664 aa, Homo sapiens
METPSQRRATRSGAQASSTPLSPTRITRLQEKEDLQELNDRLAVYIDRVRSLETENAGLRLRITESEEVVSREVSGIKAAYEAELGDARKTLDSVAKERARLQLELSKVREEFKELKARNTKKEGDLIAAQARLKDLEALLNSKEAALSTALSEKRTLEGELHDLRGQVAKLEAALGEAKKQLQDEMLRRVDAENRLQTMKEELDFQKNIYSEELRETKRRHETRLVEIDNGKQREFESRLADALQELRAQHEDQVEQYKKELEKTYSAKLDNARQSAERNSNLVGAAHEELQQSRIRIDSLSAQLSQLQKQLAAKEAKLRDLEDSLARERDTSRRLLAEKEREMAEMRARMQQQLDEYQELLDIKLALDMEIHAYRKLLEGEEERLRLSPSPTSQRSRGRASSHSSQTQGGGSVTKKRKLESTESRSSFSQHARTSGRVAVEEVDEEGKFVRLRNKSNEDQSMGNWQIKRQNGDDPLLTYRFPPKFTLKAGQVVTIWAAGAGATHSPPTDLVWKAQNTWGCGNSLRTALINSTGEEVAMRKLVRSVTVVEDDEDEDGDDLLHHHHGSHCSSSGDPAEYNLRSRTVLCGTCGQPADKASASGSGAQVGGPISSGSSASSVTVTRSYRSVGGSGGGSFGDNLVTRSYLLGNSSPRTQSPQNCSIM

SEQ ID NO: 2 - protein, 646 aa, Homo sapiens
METPSQRRATRSGAQASSTPLSPTRITRLQEKEDLQELNDRLAVYIDRVRSLETENAGLRLRITESEEVVSREVSGIKAAYEAELGDARKTLDSVAKERARLQLELSKVREEFKELKARNTKKEGDLIAAQARLKDLEALLNSKEAALSTALSEKRTLEGELHDLRGQVAKLEAALGEAKKQLQDEMLRRVDAENRLQTMKEELDFQKNIYSEELRETKRRHETRLVEIDNGKQREFESRLADALQELRAQHEDQVEQYKKELEKTYSAKLDNARQSAERNSNLVGAAHEELQQSRIRIDSLSAQLSQLQKQLAAKEAKLRDLEDSLARERDTSRRLLAEKEREMAEMRARMQQQLDEYQELLDIKLALDMEIHAYRKLLEGEEERLRLSPSPTSQRSRGRASSHSSQTQGGGSVTKKRKLESTESRSSFSQHARTSGRVAVEEVDEEGKFVRLRNKSNEDQSMGNWQIKRQNGDDPLLTYRFPPKFTLKAGQVVTIWAAGAGATHSPPTDLVWKAQNTWGCGNSLRTALINSTGEEVAMRKLVRSVTVVEDDEDEDGDDLLHHHHGSHCSSSGDPAEYNLRSRTVLCGTCGQPADKASASGSGAQVGGPISSGSSASSVTVTRSYRSVGGSGGGSFGDNLVTRSY

SEQ ID NO: 3 - DNA, 1995 bp, Homo sapiens
atggagaccccgtcccagcggcgcgccacccgcagcggggcgcaggccagctccactccgctgtcgcccacccgcatcacccggctgcaggagaaggaggacctgcaggagctcaatgatcgcttggcggtctacatcgaccgtgtgcgctcgctggaaacggagaacgcagggctgcgccttcgcatcaccgagtctgaagaggtggtcagccgcgaggtgtccggcatcaaggccgcctacgaggccgagctcggggatgcccgcaagacccttgactcagtagccaaggagcgcgcccgcctgcagctggagctgagcaaagtgcgtgaggagtttaaggagctgaaagcgcgcaataccaagaaggagggtgacctgatagctgctcaggctcggctgaaggacctggaggctctgctgaactccaaggaggccgcactgagcactgctctcagtgagaagcgcacgctggagggcgagctgcatgatctgcggggccaggtggccaagcttgaggcagccctaggtgaggccaagaagcaacttcaggatgagatgctgcggcgggtggatgctgagaacaggctgcagaccatgaaggaggaactggacttccagaagaacatctacagtgaggagctgcgtgagaccaagcgccgtcatgagacccgactggtggagattgacaatgggaagcagcgtgagtttgagagccggctggcggatgcgctgcaggaactgcgggcccagcatgaggaccaggtggagcagtataagaaggagctggagaagacttattctgccaagctggacaatgccaggcagtctgctgagaggaacagcaacctggtgggggctgcccacgaggagctgcagcagtcgcgcatccgcatcgacagcctctctgcccagctcagccagctccagaagcagctggcagccaaggaggcgaagcttcgagacctggaggactcactggcccgtgagcgggacaccagccggcggctgctggcggaaaaggagcgggagatggccgagatgcgggcaaggatgcagcagcagctggacgagtaccaggagcttctggacatcaagctggccctggacatggagatccacgcctaccgcaagctcttggagggcgaggaggagaggctacgcctgtcccccagccctacctcgcagcgcagccgtggccgtgcttcctctcactcatcccagacacagggtgggggcagcgtcaccaaaaagcgcaaactggagtccactgagagccgcagcagcttctcacagcacgcacgcactagcgggcgcgtggccgtggaggaggtggatgaggagggcaagtttgtccggctgcgcaacaagtccaatgaggaccagtccatgggcaattggcagatcaagcgccagaatggagatgatcccttgctgacttaccggttcccaccaaagttcaccctgaaggctgggcaggtggtgacgatctgggctgcaggagctggggccacccacagcccccctaccgacctggtgtggaaggcacagaacacctggggctgcgggaacagcctgcgtacggctctcatcaactccactggggaagaagtggccatgcgcaagctggtgcgctcagtgactgtggttgaggacgacgaggatgaggatggagatgacctgctccatcaccaccacggctcccactgcagcagctcgggggaccccgctgagtacaacctgcgctcgcgcaccgtgctgtgcgggacctgcgggcagcctgccgacaaggcatctgccagcggctcaggagcccaggtgggcggacccatctcctctggctcttctgcctccagtgtcacggtcactcgcagctaccgcagtgtggggggcagtgggggtggcagcttcggggacaatctggtcacccgctcctacctcctgggcaactccagcccccgaacccagagcccccagaactgcagcatcatgtaa

SEQ ID NO: 4 - protein, 572 aa, Homo sapiens
METPSQRRATRSGAQASSTPLSPTRITRLQEKEDLQELNDRLAVYIDRVRSLETENAGLRLRITESEEVVSREVSGIKAAYEAELGDARKTLDSVAKERARLQLELSKVREEFKELKARNTKKEGDLIAAQARLKDLEALLNSKEAALSTALSEKRTLEGELHDLRGQVAKLEAALGEAKKQLQDEMLRRVDAENRLQTMKEELDFQKNIYSEELRETKRRHETRLVEIDNGKQREFESRLADALQELRAQHEDQVEQYKKELEKTYSAKLDNARQSAERNSNLVGAAHEELQQSRIRIDSLSAQLSQLQKQLAAKEAKLRDLEDSLARERDTSRRLLAEKEREMAEMRARMQQQLDEYQELLDIKLALDMEIHAYRKLLEGEEERLRLSPSPTSQRSRGRASSHSSQTQGGGSVTKKRKLESTESRSSFSQHARTSGRVAVEEVDEEGKFVRLRNKSNEDQSMGNWQIKRQNGDDPLLTYRFPPKFTLKAGQVVTIWAAGAGATHSPPTDLVWKAQNTWGCGNSLRTALINSTGEEVAMRKLVRSVTVVEDDEDEDGDDLLHHHHVSGSRR

SEQ ID NO: 5 - protein, 634 aa, Homo sapiens
METPSQRRATRSGAQASSTPLSPTRITRLQEKEDLQELNDRLAVYIDRVRSLETENAGLRLRITESEEVVSREVSGIKAAYEAELGDARKTLDSVAKERARLQLELSKVREEFKELKARNTKKEGDLIAAQARLKDLEALLNSKEAALSTALSEKRTLEGELHDLRGQVAKLEAALGEAKKQLQDEMLRRVDAENRLQTMKEELDFQKNIYSEELRETKRRHETRLVEIDNGKQREFESRLADALQELRAQHEDQVEQYKKELEKTYSAKLDNARQSAERNSNLVGAAHEELQQSRIRIDSLSAQLSQLQKQLAAKEAKLRDLEDSLARERDTSRRLLAEKEREMAEMRARMQQQLDEYQELLDIKLALDMEIHAYRKLLEGEEERLRLSPSPTSQRSRGRASSHSSQTQGGGSVTKKRKLESTESRSSFSQHARTSGRVAVEEVDEEGKFVRLRNKSNEDQSMGNWQIKRQNGDDPLLTYRFPPKFTLKAGQVVTIWAAGAGATHSPPTDLVWKAQNTWGCGNSLRTALINSTGEGSHCSSSGDPAEYNLRSRTVLCGTCGQPADKASASGSGAQVGGPISSGSSASSVTVTRSYRSVGGSGGGSFGDNLVTRSYLLGNSSPRTQSPQNCSIM

SEQ ID NO: 6 - protein, 574 aa, Homo sapiens
MGNSEGCNTKKEGDLIAAQARLKDLEALLNSKEAALSTALSEKRTLEGELHDLRGQVAKLEAALGEAKKQLQDEMLRRVDAENRLQTMKEELDFQKNIYSEELRETKRRHETRLVEIDNGKQREFESRLADALQELRAQHEDQVEQYKKELEKTYSAKLDNARQSAERNSNLVGAAHEELQQSRIRIDSLSAQLSQLQKQLAAKEAKLRDLEDSLARERDTSRRLLAEKEREMAEMRARMQQQLDEYQELLDIKLALDMEIHAYRKLLEGEEERLRLSPSPTSQRSRGRASSHSSQTQGGGSVTKKRKLESTESRSSFSQHARTSGRVAVEEVDEEGKFVRLRNKSNEDQSMGNWQIKRQNGDDPLLTYRFPPKFTLKAGQVVTIWAAGAGATHSPPTDLVWKAQNTWGCGNSLRTALINSTGEEVAMRKLVRSVTVVEDDEDEDGDDLLHHHHGSHCSSSGDPAEYNLRSRTVLCGTCGQPADKASASGSGAQVGGPISSGSSASSVTVTRSYRSVGGSGGGSFGDNLVTRSYLLGNSSPRTQSPQNCSIIQEMGMRWEVEEGRRKVSLSCLP

SEQ ID NO: 7 - protein, 565 aa, Homo sapiens
MDLEAWDPHLEPDAEAMVDGNTKKEGDLIAAQARLKDLEALLNSKEAALSTALSEKRTLEGELHDLRGQVAKLEAALGEAKKQLQDEMLRRVDAENRLQTMKEELDFQKNIYSEELRETKRRHETRLVEIDNGKQREFESRLADALQELRAQHEDQVEQYKKELEKTYSAKLDNARQSAERNSNLVGAAHEELQQSRIRIDSLSAQLSQLQKQLAAKEAKLRDLEDSLARERDTSRRLLAEKEREMAEMRARMQQQLDEYQELLDIKLALDMEIHAYRKLLEGEEERLRLSPSPTSQRSRGRASSHSSQTQGGGSVTKKRKLESTESRSSFSQHARTSGRVAVEEVDEEGKFVRLRNKSNEDQSMGNWQIKRQNGDDPLLTYRFPPKFTLKAGQVVTIWAAGAGATHSPPTDLVWKAQNTWGCGNSLRTALINSTGEEVAMRKLVRSVTVVEDDEDEDGDDLLHHHHGSHCSSSGDPAEYNLRSRTVLCGTCGQPADKASASGSGAQVGGPISSGSSASSVTVTRSYRSVGGSGGGSFGDNLVTRSYLLGNSSPRTQSPQNCSIM

SEQ ID NO: 8 - protein, 614 aa, Homo sapiens
METPSQRRATRSGAQASSTPLSPTRITRLQEKEDLQELNDRLAVYIDRVRSLETENAGLRLRITESEEVVSREVSGIKAAYEAELGDARKTLDSVAKERARLQLELSKVREEFKELKARNTKKEGDLIAAQARLKDLEALLNSKEAALSTALSEKRTLEGELHDLRGQVAKLEAALGEAKKQLQDEMLRRVDAENRLQTMKEELDFQKNIYSEELRETKRRHETRLVEIDNGKQREFESRLADALQELRAQHEDQVEQYKKELEKTYSAKLDNARQSAERNSNLVGAAHEELQQSRIRIDSLSAQLSQLQKQLAAKEAKLRDLEDSLARERDTSRRLLAEKEREMAEMRARMQQQLDEYQELLDIKLALDMEIHAYRKLLEGEEERLRLSPSPTSQRSRGRASSHSSQTQGGGSVTKKRKLESTESRSSFSQHARTSGRVAVEEVDEEGKFVRLRNKSNEDQSMGNWQIKRQNGDDPLLTYRFPPKFTLKAGQVVTIWAAGAGATHSPPTDLVWKAQNTWGCGNSLRTALINSTGEEVAMRKLVRSVTVVEDDEDEDGDDLLHHHHGSHCSSSGDPAEYNLRSRTVLCGTCGQPADKASASGSGAQSPQNCSIM

SEQ ID NO: 9 - DNA, 113 bp, artificial
  oligonucleotide
tctgtgtccttcctccaacccttccaggagctgcgtgagaccaagcgacgtcatgagacccgactggtggagattgacaatgggaagcagcgtgagtttgagagccggctggc

SEQ ID NO: 10 - DNA, 20 bp, artificial
  oligonucleotide
ccaccagtcgggtctcagga

SEQ ID NO: 11 - DNA, 36 bp, artificial
  oligonucleotide
gtcagatccgctagcgctaccatggtgagcaagggc

SEQ ID NO: 12 - DNA, 22 bp, artificial
  oligonucleotide
gtctccatgctagccggtgcag

SEQ ID NO: 13 - DNA, 23 bp, artificial
  oligonucleotide
ggctagcatggagaccccgtccc

SEQ ID NO: 14 - DNA, 45 bp, artificial
  oligonucleotide
tatagggcgaattgggtaccttacatgatgctgcagttctggggg

SEQ ID NO: 15 - DNA, 30 bp, artificial
  partial sequence Fig. 1
cgtgagaccaagcgccgtcatgagacccga

SEQ ID NO: 16 - DNA, 30 bp, artificial
  partial sequence Fig. 1
cgtgagaccaagcgacgtcatgagacccga

SEQ ID NO: 17 - DNA, 12 bp, artificial
  partial sequence Fig. 1
gtcatgagaccc

SEQ ID NO: 18 - DNA, 13 bp, artificial
  partial sequence Fig. 1
gtcattgagaccc

SEQ ID NO: 19 - DNA, 9610 bp, artificial
  Plasmid vector LMNA-2A-GFP
cattcgccattcaggctgcaaataagcgttgatattcagtcaattacaaacattaataacgaagagatgacagaaaaattttcattctgtgacagagaaaaagtagccgaagatgacggtttgtcacatggagttggcaggatgtttgattaaaaacataacaggaagaaaaatgccccgctgtgggcggacaaaatagttgggaactgggaggggtggaaatggagtttttaaggattatttagggaagagtgacaaaatagatgggaactgggtgtagcgtcgtaagctaatacgaaaattaaaaatgacaaaatagtttggaactagatttcacttatctggttcggatctcctaggcgatatcagtgatcagatccagacatgataagatacattgatgagtttggacaaaccacaactagaatgcagtgaaaaaaatgctttatttgtgaaatttgtgatgctattgctttatttgtaaccattataagctgcaataaacaagttaacttacttgtacagctcgtccatgccgagagtgatcccggcggcggtcacgaactccagcaggaccatgtgatcgcgcttctcgttggggtctttgctcagggcggactgggtgctcaggtagtggttgtcgggcagcagcacggggccgtcgccgatgggggtgttctgctggtagtggtcggcgagctgcacgctgccgtcctcgatgttgtggcggatcttgaagttcaccttgatgccgttcttctgcttgtcggccatgatatagacgttgtggctgttgtagttgtactccagcttgtgccccaggatgttgccgtcctccttgaagtcgatgcccttcagctcgatgcggttcaccagggtgtcgccctcgaacttcacctcggcgcgggtcttgtagttgccgtcgtccttgaagaagatggtgcgctcctggacgtagccttcgggcatggcggacttgaagaagtcgtgctgcttcatgtggtcggggtagcggctgaagcactgcacgccgtaggtcagggtggtcacgagggtgggccagggcacgggcagcttgccggtggtgcagatgaacttcagggtcagcttgccgtaggtggcatcgccctcgccctcgccggacacgctgaacttgtggccgtttacgtcgccgtccagctcgaccaggatgggcaccaccccggtgaacagctcctcgcccttgctcaccatgctagcgtttaaattgtgtaatttatgtagctgtaatttttaccttattaatattttttacgctttgcattcgacgactgaactcccaaatatatgtttaactcgtcttggtcgtttgaatttttgttgctgtgtttcctaatattttccatcaccttaaatatgttattgtaatcctcaatgttgaacttgcaattggacacggcatagttttccatagtcgtgtaaaacatggtattggctgcattgtaatacatccgactgagcgggtacggatctatgtgtttgagcagcctgttcaaaaactctgcatcgtcgcaaaacggaatttaacaacaacaattgcattcattttatgtttcaggttcagggggaggtgtgggaggttttttaaagcaagtaaaacctctacaaatgtggtatggctgattatgatcctctagtacttctcgacaagcttacagcttgcatgcctgcaggcagctgcgcgctcgctcgctcactgaggccgcccgggcaaagcccgggcgtcgggcgacctttggtcgcccggcctcagtgagcgagcgagcgcgcagagagggagtggccaactccatcactaggggttccttgtagttaatgattaacccgccatgctacttatctacgtagccatgctctagagcggccgcacgcgttcatagcccatatatggagttccgcgttacataacttacggtaaatggcccgcctggctgaccgcccaacgacccccgcccattgacgtcaataatgacgtatgttcccatagtaacgccaatagggactttccattgacgtcaatgggtggagtatttacggtaaactgcccacttggcagtacatcaagtgtatcatatgccaagtacgccccctattgacgtcaatgacggtaaatggcccgcctggcattatgcccagtacatgaccttatgggactttcctacttggcagtacatctacgtattagtcatcgctattaccatggtgatgcggttttggcagtacatcaatgggcgtggatagcggtttgactcacggggatttccaagtctccaccccattgacgtcaatgggagtttgttttggcaccaaaatcaacgggactttccaaaatgtcgtaacaactccgccccattgacgcaaatgggcggtaggcgtgtacggtgggaggtctatataagcagagctggtttagtgaaccgtcagatccgctagcgctaccatggtgagcaagggcgaggagctgttcaccggggtggtgcccatcctggtcgagctggacggcgacgtaaacggccacaagttcagcgtgtccggcgagggcgagggcgatgccacctacggcaagctgaccctgaagttcatctgcaccaccggcaagctgcccgtgccctggcccaccctcgtgaccaccctgacctacggcgtgcagtgcttcagccgctaccccgaccacatgaagcagcacgacttcttcaagtccgccatgcccgaaggctacgtccaggagcgcaccatcttcttcaaggacgacggcaactacaagacccgcgccgaggtgaagttcgagggcgacaccctggtgaaccgcatcgagctgaagggcatcgacttcaaggaggacggcaacatcctggggcacaagctggagtacaactacaacagccacaacgtctatatcatggccgacaagcagaagaacggcatcaaggtgaacttcaagatccgccacaacatcgaggacggcagcgtgcagctcgccgaccactaccagcagaacacccccatcggcgacggccccgtgctgctgcccgacaaccactacctgagcacccagtccgccctgagcaaagaccccaacgagaagcgcgatcacatggtcctgctggagttcgtgaccgccgccgggatcactctcggcatggacgagctgtacaagtactcagatctcgagctcaaggagggcagaggaagtcttctaacatgcggtgacgtggaggagaatcccggccctgcaccggctagcatggagaccccgtcccagcggcgcgccacccgcagcggggcgcaggccagctccactccgctgtcgcccacccgcatcacccggctgcaggagaaggaggacctgcaggagctcaatgatcgcttggcggtctacatcgaccgtgtgcgctcgctggaaacggagaacgcagggctgcgccttcgcatcaccgagtctgaagaggtggtcagccgcgaggtgtccggcatcaaggccgcctacgaggccgagctcggggatgcccgcaagacccttgactcagtagccaaggagcgcgcccgcctgcagctggagctgagcaaagtgcgtgaggagtttaaggagctgaaagcgcgcaataccaagaaggagggtgacctgatagctgctcaggctcggctgaaggacctggaggctctgctgaactccaaggaggccgcactgagcactgctctcagtgagaagcgcacgctggagggcgagctgcatgatctgcggggccaggtggccaagcttgaggcagccctaggtgaggccaagaagcaacttcaggatgagatgctgcggcgggtggatgctgagaacaggctgcagaccatgaaggaggaactggacttccagaagaacatctacagtgaggagctgcgtgagaccaagcgccgtcatgagacccgactggtggagattgacaatgggaagcagcgtgagtttgagagccggctggcggatgcgctgcaggaactgcgggcccagcatgaggaccaggtggagcagtataagaaggagctggagaagacttattctgccaagctggacaatgccaggcagtctgctgagaggaacagcaacctggtgggggctgcccacgaggagctgcagcagtcgcgcatccgcatcgacagcctctctgcccagctcagccagctccagaagcagctggcagccaaggaggcgaagcttcgagacctggaggactcactggcccgtgagcgggacaccagccggcggctgctggcggaaaaggagcgggagatggccgagatgcgggcaaggatgcagcagcagctggacgagtaccaggagcttctggacatcaagctggccctggacatggagatccacgcctaccgcaagctcttggagggcgaggaggagaggctacgcctgtcccccagccctacctcgcagcgcagccgtggccgtgcttcctctcactcatcccagacacagggtgggggcagcgtcaccaaaaagcgcaaactggagtccactgagagccgcagcagcttctcacagcacgcacgcactagcgggcgcgtggccgtggaggaggtggatgaggagggcaagtttgtccggctgcgcaacaagtccaatgaggaccagtccatgggcaattggcagatcaagcgccagaatggagatgatcccttgctgacttaccggttcccaccaaagttcaccctgaaggctgggcaggtggtgacgatctgggctgcaggagctggggccacccacagcccccctaccgacctggtgtggaaggcacagaacacctggggctgcgggaacagcctgcgtacggctctcatcaactccactggggaagaagtggccatgcgcaagctggtgcgctcagtgactgtggttgaggacgacgaggatgaggatggagatgacctgctccatcaccaccacggctcccactgcagcagctcgggggaccccgctgagtacaacctgcgctcgcgcaccgtgctgtgcgggacctgcgggcagcctgccgacaaggcatctgccagcggctcaggagcccaggtgggcggacccatctcctctggctcttctgcctccagtgtcacggtcactcgcagctaccgcagtgtggggggcagtgggggtggcagcttcggggacaatctggtcacccgctcctacctcctgggcaactccagcccccgaacccagagcccccagaactgcagcatcatgtaaggtacccaattcgccctatagtgagtcgtattacgcgcgcagcggccgaccatggcccaacttgtttattgcagcttataatggttacaaataaagcaatagcatcacaaatttcacaaataaagcatttttttcactgcattctagttgtggtttgtccaaactcatcaatgtatcttatcatgtctggatctccggaccacgtgcggaccgagcggccgctctagagcatggctacgtagataagtagcatggcgggttaatcattaactacaaggaacccctagtgatggagttggccactccctctctgcgcgctcgctcgctcactgaggccgggcgaccaaaggtcgcccgacgcccgggctttgcccgggcggcctcagtgagcgagcgagcgcgcagctgcctgcaggtctgagacaataaccctgataaatgcttcaataatgtagccaaccactagaactatagctagagtcctgggcgaacaaacgatgctcgccttccagaaaaccgaggatgcgaaccacttcatccggggtcagcaccaccggcaagcgccgcgacggccgaggtcttccgatctcctgaagccagggcagatccgtgcacagcaccttgccgtagaagaacagcaaggccgccaatgcctgacgatgcgtggagaccgaaaccttgcgctcgttcgccagccaggacagaaatgcctcgacttcgctgctgcccaaggttgccgggtgacgcacaccgtggaaacggatgaaggcacgaacccagttgacataagcctgttcggttcgtaaactgtaatgcaagtagcgtatgcgctcacgcaactggtccagaaccttgaccgaacgcagcggtggtaacggcgcagtggcggttttcatggcttgttatgactgtttttttgtacagtctatgcctcgggcatccaagcagcaagcgcgttacgccgtgggtcgatgtttgatgttatggagcagcaacgatgttacgcagcagcaacgatgttacgcagcagggcagtcgccctaaaacaaagttaggtggctcaagtatgggcatcattcgcacatgtaggctcggccctgaccaagtcaaatccatgcgggctgctcttgatcttttcggtcgtgagttcggagacgtagccacctactcccaacatcagccggactccgattacctcgggaacttgctccgtagtaagacattcatcgcgcttgctgccttcgaccaagaagcggttgttggcgctctcgcggcttacgttctgcccaggtttgagcagccgcgtagtgagatctatatctatgatctcgcagtctccggcgagcaccggaggcagggcattgccaccgcgctcatcaatctcctcaagcatgaggccaacgcgcttggtgcttatgtgatctacgtgcaagcagattacggtgacgatcccgcagtggctctctatacaaagttgggcatacgggaagaagtgatgcactttgatatcgacccaagtaccgccacctaacaattcgttcaagccgagatcggcttcccggccgcggagttgttcggtaaattgtcacaacgccgcgaatatagtctttaccatgcccttggccacgcccctctttaatacgacgggcaatttgcacttcagaaaatgaagagtttgctttagccataacaaaagtccagtatgctttttcacagcataactggactgatttcagtttacaactattctgtctagtttaagactttattgtcatagtttagatctattttgttcagtttaagactttattgtccgcccacacccgcttacgcagggcatccatttattactcaaccgtaaccgattttgccaggttacgcggctggtctgcggtgtgaaataccgcacagatgcgtaaggagaaaataccgcatcaggcgctcttccgcttcctcgctcactgactcgctgcgctcggtcgttcggctgcggcgagcggtatcagctcactcaaaggcggtaatacggttatccacagaatcaggggataacgcaggaaagaacatgtgagcaaaaggccagcaaaaggccaggaaccgtaaaaaggccgcgttgctggcgtttttccataggctccgcccccctgacgagcatcacaaaaatcgacgctcaagtcagaggtggcgaaacccgacaggactataaagataccaggcgtttccccctggaagctccctcgtgcgctctcctgttccgaccctgccgcttaccggatacctgtccgcctttctcccttcgggaagcgtggcgctttctcaatgctcacgctgtaggtatctcagttcggtgtaggtcgttcgctccaagctgggctgtgtgcacgaaccccccgttcagcccgaccgctgcgccttatccggtaactatcgtcttgagtccaacccggtaagacacgacttatcgccactggcagcagccactggtaacaggattagcagagcgaggtatgtaggcggtgctacagagttcttgaagtggtggcctaactacggctacactagaaggacagtatttggtatctgcgctctgctgaagccagttaccttcggaaaaagagttggtagctcttgatccggcaaacaaaccaccgctggtagcggtggtttttttgtttgcaagcagcagattacgcgcagaaaaaaaggatctcaagaagatcctttgatcttttctacggggtctgacgctcagtggaacgaaaactcacgttaagggattttggtcatgagattatcaaaaaggatcttcacctagatccttttaaattaaaaatgaagttttaaatcaatctaaagtatatatgagtaaacttggtctgacagttaccaatgcttaatcagtgaggcacctatctcagcgatctgtctatttcgttcatccatagttgcctgactccccgtcgtgtagataactacgatacgggagggcttaccatctggccccagtgctgcaatgataccgcgagacccacgctcaccggctccagatttatcagcaataaaccagccagccggaagggccgagcgcagaagtggtcctgcaactttatccgcctccatccagtctattaattgttgccgggaagctagagtaagtagttcgccagttaatagtttgcgcaacgttgttgccattgctacaggcatcgtggtgtcacgctcgtcgtttggtatggcttcattcagctccggttcccaacgatcaaggcgagttacatgatcccccatgttgtgcaaaaaagcggttagctccttcggtcctccgatcgttgtcagaagtaagttggccgcagtgttatcactcatggttatggcagcactgcataattctcttactgtcatgccatccgtaagatgcttttctgtgactggtgagtactcaaccaagtcattctgagaatagtgtatgcggcgaccgagttgctcttgcccggcgtcaatacgggataataccgcgccacatagcagaactttaaaagtgctcatcattggaaaacgttcttcggggcgaaaactctcaaggatcttaccgctgttgagatccagttcgatgtaacccactcgtgcacccaactgatcttcagcatcttttactttcaccagcgtttctgggtgagcaaaaacaggaaggcaaaatgccgcaaaaaagggaataagggcgacacggaaatgttgaatactcatactcttcctttttcaatattattgaagcatttatcagggttattgtctcatgagcggatacatatttgaatgtatttagaaaaataaacaaataggggttccgcgcacatttccccgaaaagtgccacctgaaattgtaaacgttaatattttgttaaaattcgcgttaaatttttgttaaatcagctcattttttaaccaataggccgaaatcggcaaaatcccttataaatcaaaagaatagaccgagatagggttgagtgttgttccagtttggaacaagagtccactattaaagaacgtggactccaacgtcaaagggcgaaaaaccgtctatcagggcgatggcccactacgtgaaccatcaccctaatcaagttttttggggtcgaggtgccgtaaagcactaaatcggaaccctaaagggagcccccgatttagagcttgacggggaaagccggcgaacgtggcgagaaaggaagggaagaaagcgaaaggagcgggcgctagggcgctggcaagtgtagcggtcacgctgcgcgtaaccaccacacccgccgcgcttaatgcgccgctacagggcgcgtc